European Patent Application EP 4 467 563 A1, published November 27, 2024. Title: LDLR derived polypeptides for antiviral uses. Applicant: JLP Health GmbH. Application DE. The sequence listing filed with the application follows.

SEQUENCE LISTING (114 sequences)

SEQ ID NO: 1 - RNA, 21 nt, synthetic construct
  source 1..21: mol_type = other RNA; note = LDLR guide RNA
gatgaacaggatccaccacga

SEQ ID NO: 2 - DNA, 18 bp, synthetic construct
  source 1..18: mol_type = other DNA; note = LDLR forward primer
ctaaccagttcctgaagc

SEQ ID NO: 3 - DNA, 18 bp, synthetic construct
  source 1..18: mol_type = other DNA; note = LDLR reverse primer
gcacccagcttgacagag

SEQ ID NO: 4 - DNA, 27 bp, synthetic construct
  source 1..27: mol_type = other DNA; note = CCHFV L Fwd
gccaactgtgackgtkttctayatgct

SEQ ID NO: 5 - DNA, 25 bp, synthetic construct
  source 1..25: mol_type = other DNA; note = CCHFV L Rev1
cggaaagcctataaaacctaccttc

SEQ ID NO: 6 - DNA, 25 bp, synthetic construct
  source 1..25: mol_type = other DNA; note = CCHFV L Rev2
cggaaagcctataaaacctgccytc

SEQ ID NO: 7 - DNA, 25 bp, synthetic construct
  source 1..25: mol_type = other DNA; note = CCHFV L Rev3
cggaaagcctaaaaaatctgccttc

SEQ ID NO: 8 - DNA, 17 bp, synthetic construct
  source 1..17: mol_type = other DNA; note = CCHFV L Probe
  misc_feature 1: note = FAM labeling
  misc_feature 17: note = MGB labeling
ctgacaagytcagcaac

SEQ ID NO: 9 - DNA, 25 bp, synthetic construct
  source 1..25: mol_type = other DNA; note = VSV M Fwd
tgatacagtacaattattttgggac

SEQ ID NO: 10 - DNA, 24 bp, synthetic construct
  source 1..24: mol_type = other DNA; note = VSV M Rev
gagactttctgttacgggatctgg

SEQ ID NO: 11 - DNA, 17 bp, synthetic construct
  source 1..17: mol_type = other DNA; note = VSV M Probe
  misc_feature 1: note = FAM labeling
  misc_feature 17: note = MGB labeling
atgatgcatgatccagc

SEQ ID NO: 12 - DNA, 19 bp, synthetic construct
  source 1..19: mol_type = other DNA; note = RNase P Fwd
agatttggacctgcgagcg

SEQ ID NO: 13 - DNA, 20 bp, synthetic construct
  source 1..20: mol_type = other DNA; note = RNase P Rev
gagcggctgtctccacaagt

SEQ ID NO: 14 - DNA, 23 bp, synthetic construct
  source 1..23: mol_type = other DNA; note = RNase P Probe
  misc_feature 1: note = FAM labeling
  misc_feature 23: note = MGB labeling
ttctgacctgaaggctctgcgcg

SEQ ID NO: 15 - DNA, 27 bp, synthetic construct
  source 1..27: mol_type = other DNA; note = CCHFV FWD
gccaactgtgackgtkttctayatgct

SEQ ID NO: 16 - DNA, 25 bp, synthetic construct
  source 1..25: mol_type = other DNA; note = CCHFV REV
cggaaagcctaaaaaatctgccttc

SEQ ID NO: 17 - DNA, 17 bp, synthetic construct
  source 1..17: mol_type = other DNA; note = CCHFV PROBE
  misc_feature 1: note = FAM labeling
  misc_feature 17: note = MGB labeling
ctgacaagytcagcaac

SEQ ID NO: 18 - protein, 767 aa, Homo sapiens
  source 1..767: note = LDLR ECTODOMAIN
AVGDRCERNEFQCQDGKCISYKWVCDGSAECQDGSDESQETCLSVTCKSGDFSCGGRVNRCIPQFWRCDGQVDCDNGSDEQGCPPKTCSQDEFRCHDGKCISRQFVCDSDRDCLDGSDEASCPVLTCGPASFQCNSSTCIPQLWACDNDPDCEDGSDEWPQRCRGLYVFQGDSSPCSAFEFHCLSGECIHSSWRCDGGPDCKDKSDEENCAVATCRPDEFQCSDGNCIHGSRQCDREYDCKDMSDEVGCVNVTLCEGPNKFKCHSGECITLDKVCNMARDCRDWSDEPIKECGTNECLDNNGGCSHVCNDLKIGYECLCPDGFQLVAQRRCEDIDECQDPDTCSQLCVNLEGGYKCQCEEGFQLDPHTKACKAVGSIAYLFFTNRHEVRKMTLDRSEYTSLIPNLRNVVALDTEVASNRIYWSDLSQRMICSTQLDRAHGVSSYDTVISRDIQAPDGLAVDWIHSNIYWTDSVLGTVSVADTKGVKRKTLFRENGSKPRAIVVDPVHGFMYWTDWGTPAKIKKGGLNGVDIYSLVTENIQWPNGITLDLLSGRLYWVDSKLHSISSIDVNGGNRKTILEDEKRLAHPFSLAVFEDKVFWTDIINEAIFSANRLTGSDVNLLAENLLSPEDMVLFHNLTQPRGVNWCERTTLSNGGCQYLCLPAPQINPHSPKFTCACPDGMLLARDMRSCLTEAEAAVATQETSTVRLKVSSTAVRTQHTTTRPVPDTSRLPGATPGLTTVEIVTMSHQALGDVAGRGNEKKPSSVR

SEQ ID NO: 19 - protein, 41 aa, Homo sapiens
  source 1..41: note = LA1
DRCERNEFQCQDGKCISYKWVCDGSAECQDGSDESQETCLS

SEQ ID NO: 20 - protein, 41 aa, Homo sapiens
  source 1..41: note = LA2
VTCKSGDFSCGGRVNRCIPQFWRCDGQVDCDNGSDEQGCPP

SEQ ID NO: 21 - protein, 39 aa, Homo sapiens
  source 1..39: note = LA3
KTCSQDEFRCHDGKCISRQFVCDSDRDCLDGSDEASCPV

SEQ ID NO: 22 - protein, 41 aa, Homo sapiens
  source 1..41: note = LA4
LTCGPASFQCNSSTCIPQLWACDNDPDCEDGSDEWPQRCRG

SEQ ID NO: 23 - protein, 39 aa, Homo sapiens
  source 1..39: note = LA5
SPCSAFEFHCLSGECIHSSWRCDGGPDCKDKSDEENCAV

SEQ ID NO: 24 - protein, 39 aa, Homo sapiens
  source 1..39: note = LA6
ATCRPDEFQCSDGNCIHGSRQCDREYDCKDMSDEVGCVN

SEQ ID NO: 25 - protein, 40 aa, Homo sapiens
  source 1..40: note = LA7
TLCEGPNKFKCHSGECITLDKVCNMARDCRDWSDEPIKEC

SEQ ID NO: 26 - protein, 40 aa, Homo sapiens
  source 1..40: note = EGFA
GTNECLDNNGGCSHVCNDLKIGYECLCPDGFQLVAQRRCE

SEQ ID NO: 27 - protein, 40 aa, Homo sapiens
  source 1..40: note = EGFB
DIDECQDPDTCSQLCVNLEGGYKCQCEEGFQLDPHTKACK

SEQ ID NO: 28 - protein, 42 aa, Homo sapiens
  source 1..42: note = LB1
SIAYLFFTNRHEVRKMTLDRSEYTSLIPNLRNVVALDTEVAS

SEQ ID NO: 29 - protein, 47 aa, Homo sapiens
  source 1..47: note = LB2
NRIYWSDLSQRMICSTQLDRAHGVSSYDTVISRDIQAPDGLAVDWIH

SEQ ID NO: 30 - protein, 43 aa, Homo sapiens
  source 1..43: note = LB3
SNIYWTDSVLGTVSVADTKGVKRKTLFRENGSKPRAIVVDPVH

SEQ ID NO: 31 - protein, 44 aa, Homo sapiens
  source 1..44: note = LB4
GFMYWTDWGTPAKIKKGGLNGVDIYSLVTENIQWPNGITLDLLS

SEQ ID NO: 32 - protein, 43 aa, Homo sapiens
  source 1..43: note = LB5
GRLYWVDSKLHSISSIDVNGGNRKTILEDEKRLAHPFSLAVFE

SEQ ID NO: 33 - protein, 43 aa, Homo sapiens
  source 1..43: note = LB6
DKVFWTDIINEAIFSANRLTGSDVNLLAENLLSPEDMVLFHNL

SEQ ID NO: 34 - protein, 262 aa, Homo sapiens
  source 1..262: note = PROP
SIAYLFFTNRHEVRKMTLDRSEYTSLIPNLRNVVALDTEVASNRIYWSDLSQRMICSTQLDRAHGVSSYDTVISRDIQAPDGLAVDWIHSNIYWTDSVLGTVSVADTKGVKRKTLFRENGSKPRAIVVDPVHGFMYWTDWGTPAKIKKGGLNGVDIYSLVTENIQWPNGITLDLLSGRLYWVDSKLHSISSIDVNGGNRKTILEDEKRLAHPFSLAVFEDKVFWTDIINEAIFSANRLTGSDVNLLAENLLSPEDMVLFHNL

SEQ ID NO: 35 - protein, 50 aa, Homo sapiens
  source 1..50: note = EGFC
GVNWCERTTLSNGGCQYLCLPAPQINPHSPKFTCACPDGMLLARDMRSCL

SEQ ID NO: 36 - protein, 48 aa, Homo sapiens
  source 1..48: note = OLSD
TQETSTVRLKVSSTAVRTQHTTTRPVPDTSRLPGATPGLTTVEIVTMS

SEQ ID NO: 37 - protein, 5 aa, synthetic construct
GGGGS

SEQ ID NO: 38 - protein, 5 aa, synthetic construct
GGSGG

SEQ ID NO: 39 - protein, 5 aa, synthetic construct
GGSSG

SEQ ID NO: 40 - protein, 5 aa, synthetic construct
GSSSG

SEQ ID NO: 41 - protein, 16 aa, synthetic construct
GGGGSLVPRGSGGGGS

SEQ ID NO: 42 - protein, 11 aa, synthetic construct
GGSGGHMGSGG

SEQ ID NO: 43 - protein, 4 aa, synthetic construct
GGAA

SEQ ID NO: 44 - protein, 6 aa, synthetic construct
GGGAAA

SEQ ID NO: 45 - protein, 10 aa, synthetic construct
GGGAAAGGAA

SEQ ID NO: 46 - protein, 8 aa, synthetic construct
AAGAATAA

SEQ ID NO: 47 - protein, 8 aa, synthetic construct
GGSGGGGG

SEQ ID NO: 48 - protein, 11 aa, synthetic construct
GGSGGSGGSGG

SEQ ID NO: 49 - protein, 11 aa, synthetic construct
GSGGGTGGGSG

SEQ ID NO: 50 - protein, 14 aa, synthetic construct
GSGGSGSGGSGGSG

SEQ ID NO: 51 - protein, 15 aa, synthetic construct
GGGGSLVPRGSGGGG

SEQ ID NO: 52 - protein, 15 aa, synthetic construct
GGGGSEAAAKGGGGS

SEQ ID NO: 53 - protein, 17 aa, synthetic construct
SRGSSGSSSSGSSGGSG

SEQ ID NO: 54 - protein, 18 aa, synthetic construct
GGGSEGGGSEGGGSEGGG

SEQ ID NO: 55 - protein, 26 aa, synthetic construct
GSGSGSGSGGSGGSGGSGGSGGSGGS

SEQ ID NO: 56 - protein, 9 aa, synthetic construct
AAGGPSGSP

SEQ ID NO: 57 - protein, 9 aa, synthetic construct
APSSGGAAP

SEQ ID NO: 58 - protein, 10 aa, synthetic construct
AAGGVPSGSP

SEQ ID NO: 59 - protein, 10 aa, synthetic construct
APSSGVGAAP

SEQ ID NO: 60 - protein, 12 aa, synthetic construct
PASGGASSPPGA

SEQ ID NO: 61 - protein, 12 aa, synthetic construct
AALGGVPSLGSP

SEQ ID NO: 62 - protein, 12 aa, synthetic construct
APSLSGVGALAP

SEQ ID NO: 63 - protein, 13 aa, synthetic construct
PASGGVASSPPGA

SEQ ID NO: 64 - protein, 15 aa, synthetic construct
PALSGGVASSPLPGA

SEQ ID NO: 65 - protein, 18 aa, synthetic construct
AAGGPSGSPAPSSGGAAP

SEQ ID NO: 66 - protein, 20 aa, synthetic construct
AAGGVPSGSPAPSSGVGAAP

SEQ ID NO: 67 - protein, 21 aa, synthetic construct
APSSGGAAPPASGGASSPPGA

SEQ ID NO: 68 - protein, 22 aa, synthetic construct
PASGGASSPPGAAAGGVPSGSP

SEQ ID NO: 69 - protein, 23 aa, synthetic construct
APSSGVGAAPPASGGVASSPPGA

SEQ ID NO: 70 - protein, 24 aa, synthetic construct
AALGGVPSLGSPAPSLSGVGALAP

SEQ ID NO: 71 - protein, 24 aa, synthetic construct
PALSGGVASSPLPGAAAGGPSGSP

SEQ ID NO: 72 - protein, 25 aa, synthetic construct
PASGGVASSPPGAAALGGVPSLGSP

SEQ ID NO: 73 - protein, 27 aa, synthetic construct
APSLSGVGALAPPALSGGVASSPLPGA

SEQ ID NO: 74 - protein, 30 aa, synthetic construct
AAGGPSGSPAPSSGGAAPPASGGASSPPGA

SEQ ID NO: 75 - protein, 31 aa, synthetic construct
APSSGGAAPPASGGASSPPGAAAGGVPSGSP

SEQ ID NO: 76 - protein, 32 aa, synthetic construct
PASGGASSPPGAAAGGVPSGSPAPSSGVGAAP

SEQ ID NO: 77 - protein, 33 aa, synthetic construct
AAGGVPSGSPAPSSGVGAAPPASGGVASSPPGA

SEQ ID NO: 78 - protein, 33 aa, synthetic construct
PALSGGVASSPLPGAAAGGPSGSPAPSSGGAAP

SEQ ID NO: 79 - protein, 35 aa, synthetic construct
APSSGVGAAPPASGGVASSPPGAAALGGVPSLGSP

SEQ ID NO: 80 - protein, 36 aa, synthetic construct
APSLSGVGALAPPALSGGVASSPLPGAAAGGPSGSP

SEQ ID NO: 81 - protein, 37 aa, synthetic construct
PASGGVASSPPGAAALGGVPSLGSPAPSLSGVGALAP

SEQ ID NO: 82 - protein, 39 aa, synthetic construct
AALGGVPSLGSPAPSLSGVGALAPPALSGGVASSPLPGA

SEQ ID NO: 83 - protein, 40 aa, synthetic construct
AAGGPSGSPAPSSGGAAPPASGGASSPPGAAAGGVPSGSP

SEQ ID NO: 84 - protein, 41 aa, synthetic construct
APSSGGAAPPASGGASSPPGAAAGGVPSGSPAPSSGVGAAP

SEQ ID NO: 85 - protein, 45 aa, synthetic construct
PASGGASSPPGAAAGGVPSGSPAPSSGVGAAPPASGGVASSPPGA

SEQ ID NO: 86 - protein, 45 aa, synthetic construct
AAGGVPSGSPAPSSGVGAAPPASGGVASSPPGAAALGGVPSLGSP

SEQ ID NO: 87 - protein, 45 aa, synthetic construct
APSLSGVGALAPPALSGGVASSPLPGAAAGGPSGSPAPSSGGAAP

SEQ ID NO: 88 - protein, 45 aa, synthetic construct
PALSGGVASSPLPGAAAGGPSGSPAPSSGGAAPPASGGASSPPGA

SEQ ID NO: 89 - protein, 47 aa, synthetic construct
APSSGVGAAPPASGGVASSPPGAAALGGVPSLGSPAPSLSGVGALAP

SEQ ID NO: 90 - protein, 48 aa, synthetic construct
AALGGVPSLGSPAPSLSGVGALAPPALSGGVASSPLPGAAAGGPSGSP

SEQ ID NO: 91 - protein, 50 aa, synthetic construct
AAGGPSGSPAPSSGGAAPPASGGASSPPGAAAGGVPSGSPAPSSGVGAAP

SEQ ID NO: 92 - protein, 52 aa, synthetic construct
PASGGVASSPPGAAALGGVPSLGSPAPSLSGVGALAPPALSGGVASSPLPGA

SEQ ID NO: 93 - protein, 54 aa, synthetic construct
APSSGGAAPPASGGASSPPGAAAGGVPSGSPAPSSGVGAAPPASGGVASSPPGA

SEQ ID NO: 94 - protein, 55 aa, synthetic construct
PALSGGVASSPLPGAAAGGPSGSPAPSSGGAAPPASGGASSPPGAAAGGVPSGSP

SEQ ID NO: 95 - protein, 57 aa, synthetic construct
PASGGASSPPGAAAGGVPSGSPAPSSGVGAAPPASGGVASSPPGAAALGGVPSLGSP

SEQ ID NO: 96 - protein, 57 aa, synthetic construct
AAGGVPSGSPAPSSGVGAAPPASGGVASSPPGAAALGGVPSLGSPAPSLSGVGALAP

SEQ ID NO: 97 - protein, 57 aa, synthetic construct
AALGGVPSLGSPAPSLSGVGALAPPALSGGVASSPLPGAAAGGPSGSPAPSSGGAAP

SEQ ID NO: 98 - protein, 57 aa, synthetic construct
APSLSGVGALAPPALSGGVASSPLPGAAAGGPSGSPAPSSGGAAPPASGGASSPPGA

SEQ ID NO: 99 - protein, 61 aa, synthetic construct
PASGGVASSPPGAAALGGVPSLGSPAPSLSGVGALAPPALSGGVASSPLPGAAAGGPSGSP

SEQ ID NO: 100 - protein, 62 aa, synthetic construct
APSSGVGAAPPASGGVASSPPGAAALGGVPSLGSPAPSLSGVGALAPPALSGGVASSPLPGA

SEQ ID NO: 101 - protein, 63 aa, synthetic construct
AAGGPSGSPAPSSGGAAPPASGGASSPPGAAAGGVPSGSPAPSSGVGAAPPASGGVASSPPGA

SEQ ID NO: 102 - protein, 65 aa, synthetic construct
PALSGGVASSPLPGAAAGGPSGSPAPSSGGAAPPASGGASSPPGAAAGGVPSGSPAPSSGVGAAP

SEQ ID NO: 103 - protein, 66 aa, synthetic construct
APSSGGAAPPASGGASSPPGAAAGGVPSGSPAPSSGVGAAPPASGGVASSPPGAAALGGVPSLGSP

SEQ ID NO: 104 - protein, 67 aa, synthetic construct
APSLSGVGALAPPALSGGVASSPLPGAAAGGPSGSPAPSSGGAAPPASGGASSPPGAAAGGVPSGSP

SEQ ID NO: 105 - protein, 69 aa, synthetic construct
PASGGASSPPGAAAGGVPSGSPAPSSGVGAAPPASGGVASSPPGAAALGGVPSLGSPAPSLSGVGALAP

SEQ ID NO: 106 - protein, 69 aa, synthetic construct
AALGGVPSLGSPAPSLSGVGALAPPALSGGVASSPLPGAAAGGPSGSPAPSSGGAAPPASGGASSPPGA

SEQ ID NO: 107 - protein, 70 aa, synthetic construct
PASGGVASSPPGAAALGGVPSLGSPAPSLSGVGALAPPALSGGVASSPLPGAAAGGPSGSPAPSSGGAAP

SEQ ID NO: 108 - protein, 71 aa, synthetic construct
APSSGVGAAPPASGGVASSPPGAAALGGVPSLGSPAPSLSGVGALAPPALSGGVASSPLPGAAAGGPSGSP

SEQ ID NO: 109 - protein, 72 aa, synthetic construct
AAGGVPSGSPAPSSGVGAAPPASGGVASSPPGAAALGGVPSLGSPAPSLSGVGALAPPALSGGVASSPLPGA

SEQ ID NO: 110 - protein, 49 aa, Homo sapiens
  source 1..49: note = LA4X
LTCGPASFQCNSSTCIPQLWACDNDPDCEDGSDEWPQRCRGLYVFQGDS

SEQ ID NO: 111 - protein, 40 aa, Homo sapiens
  source 1..40: note = LA6X
ATCRPDEFQCSDGNCIHGSRQCDREYDCKDMSDEVGCVNV

SEQ ID NO: 112 - protein, 43 aa, Homo sapiens
  source 1..43: note = EGFBX
DIDECQDPDTCSQLCVNLEGGYKCQCEEGFQLDPHTKACKAVG

SEQ ID NO: 113 - protein, 266 aa, Homo sapiens
  source 1..266: note = PROPX
SIAYLFFTNRHEVRKMTLDRSEYTSLIPNLRNVVALDTEVASNRIYWSDLSQRMICSTQLDRAHGVSSYDTVISRDIQAPDGLAVDWIHSNIYWTDSVLGTVSVADTKGVKRKTLFRENGSKPRAIVVDPVHGFMYWTDWGTPAKIKKGGLNGVDIYSLVTENIQWPNGITLDLLSGRLYWVDSKLHSISSIDVNGGNRKTILEDEKRLAHPFSLAVFEDKVFWTDIINEAIFSANRLTGSDVNLLAENLLSPEDMVLFHNLTQPR

SEQ ID NO: 114 - protein, 58 aa, Homo sapiens
  source 1..58: note = EGFCX
GVNWCERTTLSNGGCQYLCLPAPQINPHSPKFTCACPDGMLLARDMRSCLTEAEAAVA